European Patent Specification EP 3 875 481 B1, published January 22, 2025. Title: NEUTRALIZING ANTIBODIES TO EBOLA VIRUS GLYCOPROTEIN AND THEIR USE. Applicant: The United States of America,  as Represented by the Secretary, Department of Health and Human Services Sullivan, Nancy Mulangu, Sabue Corti, Davide Lanzavecchia, Antonia Graham, Barney Muyembe-Tamfun, Jean-Jacques Trefry, John Ledgerwood, Julie Stanley, Daphne. The sequence listing filed with the application follows.

SEQUENCE LISTING (66 sequences)

SEQ ID NO: 1 - protein, 119 aa, homo sapiens [sequence omitted]

SEQ ID NO: 2 - protein, 107 aa, homo sapiens [sequence omitted]

SEQ ID NO: 3 - protein, 125 aa, homo sapiens
QVQLQESGPGLVKPSDTLSLTCTVSGGSLSSFYWSWIRQPPGKGLEWIGYIYYSGSPNYSPSLESRVTMSVDTTRNQISLKLDSVTAADTAVYYCVRASRSYYWGSYRPTAFDSWGQGTLVTVSS

SEQ ID NO: 4 - protein, 105 aa, homo sapiens
SYELTQPLSVSVSPGQTAIFTCSGDNLGDKYVCWFQQRPGQSPMLLIYQDNKRPSGIPERFSGSNSGNTATLTISGTQSTDEADYYCQTWDSTVVFGGGTKLTVL

SEQ ID NO: 5 - protein, 123 aa, homo sapiens
QVQLVQSGAEVKKPGSSVKVSCKTSGGTLSNYAISWVRQAPGQGLEWMGGTIPTLGMSTYAPNFQGRVAITADKSTSTAYMELSSLRSDDTAVYYCATMGSADTSFYFYMDVWGKGTTVTVSS

SEQ ID NO: 6 - protein, 108 aa, homo sapiens
EIVLTQSPGTLSLSPGERATLSCRASQSVSSSYLAWYQQKPGQAPRLLIYGTSSRATGIPDRFSGSASGTDFTLTISRLEPEDFAVYYCQQYAYSPFTFGPGTKVDIK

SEQ ID NO: 7 - DNA, 358 bp, homo sapiens
gaggtgcagctggtggagtctgggggaggtttaattcagccgggggggtccctgagactctcctgtgcagcctctggattcgccctcagaatgtacgacatgcactgggtccgtcagacaatagataaacgtctcgagtgggtctcagctgtgggtccttctggtgacacctactatgcagactccgtgaagggccgattcgccgtctccagagagaatgccaagaactccttgtctcttcagatgaacagcctgacagccggggacacggctatatactattgtgtaaggtctgaccgaggagtggctggcctttttgacagctggggccagggaatcctggtcaccgtctcttcag

SEQ ID NO: 8 - DNA, 322 bp, homo sapiens
gacatccagatgacccagtctccatcatccctgtctgcatctgtgggagacagaatcaccatcacttgccgggcgagtcaggcctttgacaattatgtagcctggtatcaacagagaccagggaaggttcctaagctcctgatctctgctgcatccgctttgcacgcaggggtcccatctcgcttcagcggcagtggctctgggacacatttcactctcaccatcagcagcctgcagcctgaagatgttgcaacttattactgtcaaaactataacagtgccccgctcactttcggcggagggaccaaggtggagatcaaac

SEQ ID NO: 9 - DNA, 376 bp, homo sapiens
caggtgcagctgcaggagtcgggcccaggactggtgaagccttcggataccctgtccctcacctgtactgtctctggtggctccctcagtagtttctactggagctggatccggcagcccccagggaagggactggagtggattgggtatatctattacagtgggagccccaactacagcccctccctcgagagtcgagtcaccatgtcagtagacacgaccaggaaccagatctccctgaagttggactctgtgaccgcggcggacacggccgtgtattactgtgtgagagcctcccgaagttactattgggggagttatcgcccaacggcttttgactcctggggccagggaaccctggtcaccgtctcctcag

SEQ ID NO: 10 - DNA, 316 bp, homo sapiens
tcctatgagctgactcagccactctcagtgtccgtgtccccaggccagacagccatcttcacctgctctggagataatttgggggataagtatgtttgctggtttcaacagaggccaggccagtcccctatgctgctcatctatcaagacaataagcggccctcggggatccctgagcgattctctggctccaactctgggaacacagccactctgactatcagcgggacccagtctacagatgaggctgactattactgtcagacgtgggacagcaccgtggtgttcggcggagggaccaaactgaccgtcctgg

SEQ ID NO: 11 - DNA, 370 bp, homo sapiens
caggtccagctggtgcagtctggggctgaggtgaagaagcctgggtcctcggtgaaagtctcctgcaagacttctggaggcaccctcagcaactatgctatcagctgggtgcgacaggcccctggacaagggcttgagtggatgggaggcaccattcctacccttggtatgtccacctacgcaccgaacttccagggcagagtcgcgattaccgcggacaaatccacgagcacagcctacatggagttgagtagtctgaggtctgacgacacggccgtttattattgtgcgactatgggcagtgcggacactagtttctacttctacatggacgtctggggcaaagggaccacggtcaccgtctcctcag

SEQ ID NO: 12 - DNA, 325 bp, homo sapiens
gaaattgtgttgacgcagtctccaggcaccctgtctttgtctccaggggagagagccaccctctcctgcagggccagtcagagtgttagtagcagctacttagcctggtaccagcagaaacctggccaggctcccagactcctcatctatggtacatccagcagggccactggcatcccagacaggttcagtggcagtgcgtctgggacagacttcactctcaccatcagcagactggagcctgaagattttgcagtgtattactgtcagcagtatgcttactcaccattcactttcggccctgggaccacagtggatatcaaac

SEQ ID NO: 13 - protein, 676 aa, Ebola virus
MVTSGILQLPRERFRKTSFFVWVIILFHKVFPIPLGVVHNNTLQVSDIDKLVCRDKLSSTSQLKSVGLNLEGNGVATDVPTATKRWGFRAGVPPKVVNYEAGEWAENCYNLDIKKADGSECLPEAPEGVRGFPRCRYVHKVSGTGPCPEGYAFHKEGAFFLYDRLASTIIYRSTTFSEGVVAFLILPETKKDFFQSPPLHEPANMTTDPSSYYHTVTLNYVADNFGTNMTNFLFQVDHLTYVQLEPRFTPQFLVQLNETIYTNGRRSNTTGTLIWKVNPTVDTGVGEWAFWENKKNFTKTLSSEELSVIFVPRAQDPGSNQKTKVTPTSFANNQTSKNHEDLVPEDPASVVQVRDLQRENTVPTPPPDTVPTTLIPDTMEEQTTSHYEPPNISRNHQERNNTAHPETLANNPPDNTTPSTPPQDGERTSSHTTPSPRPVPTSTIHPTTRETHIPTTMTTSHDTDSNRPNPIDISESTEPGPLTNTTRGAANLLTGSRRTRREITLRTQAKCNPNLHYWTTQDEGAAIGLAWIPYFGPAAEGIYTEGIMHNQNGLICGLRQLANETTQALQLFLRATTELRTFSILNRKAIDFLLQRWGGTCHILGPDCCIEPHDWTKNITDKIDQIIHDFIDKPLPDQTDNDNWWTGWRQWVPAGIGITGVIIAVIALLCICKFLL

SEQ ID NO: 14 - protein, 676 aa, Ebola virus
MEGLSLLQLPRDKFRKSSFFVWVIILFQKAFSMPLGVVTNSTLEVTEIDQLVCKDHLASTDQLKSVGLNLEGSGVSTDIPSATKRWGFRSGVPPKVFSYEAGEWAENCYNLEIKKPDGSECLPPPPDGVRGFPRCRYVHKAQGTGPCPGDYAFHKDGAFFLYDRLASTVIYRGVNFAEGVIAFLILAKPKETFLQSPPIREAVNYTENTSSYYATSYLEYEIENFGAQHSTTLFKINNNTFVLLDRPHTPQFLFQLNDTIHLHQQLSNTTGKLIWTLDANINADIGEWAFWENKKNLSEQLRGEELSFETLSLNETEDDDATSSRTTKGRISDRATRKYSDLVPKDSPGMVSLHVPEGETTLPSQNSTEGRRVDVNTQETITETTATIIGTNGNNMQISTIGTGLSSSQILSSSPTMAPSPETQTSTTYTPKLPVMTTEESTTPPRNSPGSTTEAPTLTTPENITTAVKTVLPQESTSNGLITSTVTGILGSLGLRKRSRRQVNTRATGKCNPNLHYWTAQEQHNAAGIAWIPYFGPGAEGIYTEGLMHNQNALVCGLRQLANETTQALQLFLRATTELRTYTILNRKAIDFLLRRWGGTCRILGPDCCIEPHDWTKNITDKINQIIHDFIDNPLPNQDNDDNWWTGWRQWIPAGIGITGIIIAIIALLCVCKLLC

SEQ ID NO: 15 - protein, 676 aa, Ebola virus
MGVTGILQLPRDRFKKTSFFLWVIILFQRTFSIPLGVIHNSTLQVSDVDKLVCRDKLSSTNQLRSVGLNLEGNGVATDVPSATKRWGFRSGVPPKVVNYEAGEWAENCYNLEIKKPDGSECLPAAPDGIRGFPRCRYVHKVSGTGPCAGDFAFHKEGAFFLYDRLASTVIYRGTTFAEGVVAFLILPQAKKDFFSSHPLREPVNATEDPSSGYYSTTIRYQATGFGTNETEYLFEVDNLTYVQLESRFTPQFLLQLNETIYTSGKRSNTTGKLIWKVNPEIDTTIGEWAFWETKKNLTRKIRSEELSFTAVSNRAKNISGQSPARTSSDPGTNTTTEDHKIMASENSSAMVQVHSQGREAAVSHLTTLATISTSPQPPTTKPGPDNSTHNTPVYKLDISEATQAEQHHRRTDNDSTTSDTPPAMTAAGPPKAENTNTSKGTDLPDPATTTSPQNHSETAGNNNTHHQDTGEESASSGKLGLITNTIAGVAGLITGGRRTRREAIVNAQPKCNPNLHYWTTQDEGAAIGLAWIPYFGPAAEGIYTEGLMHNQDGLICGLRQLANETTQALQLFLRATTELRTFSILNRKAIDFLLQRWGGTCHILGPDCCIEPHDWTKNITDKIDQIIHDFVDKTLPDQGDNDNWWTGWRQWIPAGIGVTGVIIAVIALFCICKFVF

SEQ ID NO: 16 - protein, 677 aa, Ebola virus
MGSGYQLLQLPRERFRKTSFLVWVIILFQRAISMPLGIVTNSTLKATEIDQLVCRDKLSSTSQLKSVGLNLEGNGIATDVPSATKRWGFRSGVPPKVVSYEAGEWAENCYNLEIKKSDGSECLPLPPDGVRGFPRCRYVHKVQGTGPCPGDLAFHKNGAFFLYDRLASTVIYRGTTFTEGVVAFLILSEPKKHFWKATPAHEPVNTTDDSTSYYMTLTLSYEMSNFGGKESNTLFKVDNHTYVQLDRPHTPQFLVQLNETLRRNNRLSNSTGRLTWTLDPKIEPDVGEWAFWETKKNFSQQLHGENLHFQILSTHTNNSSDQSPAGTVQGKISYHPPTNNSELVPTDSPPVVSVLTAGRTEEMSTQGLTNGETITGFTANPMTTTIAPSPTMTSEVDNNVPSEQPNNTASIEDSPPSASNETIDHSEMNPIQGSNNSAQSPQTKTTPAPTASPMTQDPQETANSSKLGTSPGSAAEPSQPGFTINTVSKVADSLSPTRKQKRSVRQNTANKCNPDLHYWTAVDEGAAVGLAWIPYFGPAAEGIYIEGVMHNQNGLICGLRQLANETTQALQLFLRATTELRTYSLLNRKAIDFLLQRWGGTCRILGPSCCIEPHDWTKNITDEINQIKHDFIDNPLPDHGDDLNLWTGWRQWIPAGIGIIGVIIAIIALLCICKILC

SEQ ID NO: 17 - protein, 676 aa, Ebola virus
MGASGILQLPRERFRKTSFFVWVIILFHKVFSIPLGVVHNNTLQVSDIDKFVCRDKLSSTSQLKSVGLNLEGNGVATDVPTATKRWGFRAGVPPKVVNCEAGEWAENCYNLAIKKVDGSECLPEAPEGVRDFPRCRYVHKVSGTGPCPGGLAFHKEGAFFLYDRLASTIIYRGTTFAEGVIAFLILPKARKDFFQSPPLHEPANMTTDPSSYYHTTTINYVVDNFGTNTTEFLFQVDHLTYVQLEARFTPQFLVLLNETIYSDNRRSNTTGKLIWKINPTVDTSMGEWAFWENKKNFTKTLSSEELSFVPVPETQNQVLDTTATVSPPISAHNHAAEDHKELVSEDSTPVVQMQNIKGKDTMPTTVTGVPTTTPSPFPINARNTDHTKSFIGLEGPQEDHSTTQPAKTTSQPTNSTESTTLNPTSEPSSRGTGPSSPTVPNTTESHAELGKTTPTTLPEQHTAASAIPRAVHPDELSGPGFLTNTIRGVTNLLTGSRRKRRDVTPNTQPKCNPNLHYWTALDEGAAIGLAWIPYFGPAAEGIYTEGIMENQNGLICGLRQLANETTQALQLFLRATTELRTFSILNRKAIDFLLQRWGGTCHILGPDCCIEPQDWTKNITDKIDQIIHDFVDNNLPNQNDGSNWWTGWKQWVPAGIGITGVIIAIIALLCICKFML

SEQ ID NO: 18 - protein, 364 aa, Ebola virus
MGVTGILQLPRDRFKRTSFFLWVIILFQRTFSIPLGVIHNSTLQVSDVDKLVCRDKLSSTNQLRSVGLNLEGNGVATDVPSATKRWGFRSGVPPKVVNYEAGEWAENCYNLEIKKPDGSECLPAAPDGIRGFPRCRYVHKVSGTGPCAGDFAFHKEGAFFLYDRLASTVIYRGTTFAEGVVAFLILPQAKKDFFSSHPLREPVNATEDPSSGYYSTTIRYQATGFGTNETEYLFEVDNLTYVQLESRFTPQFLLQLNETIYTSGKRSNTTGKLIWKVNPEIDTTIGEWAFWETKKTSLEKFAVKSCLSQLYQTEPKTSVVRVRRELLPTQGPTQQLKTTKSWLQKIPLQWFKCTVKEGKLQCRI

SEQ ID NO: 19 - protein, 128 aa, homo sapiens
DVQLVESGGGVVQPGGSLKLACVVSGFRFSDYWMSWVRQAPGKGLEWVANIKQDGSGKYYVDSVKGRFTVSRDNAKNSLYLHMTSLGAEDTAVYFCARAAPTGSYTNILVDNVHFDYWGQGILVAVSS

SEQ ID NO: 20 - protein, 107 aa, homo sapiens
GIQLTQSPGSLSASVGDSVTITCRPNQNIATYINWYQQTPGKAPKLLIYAASILQSGVPSRFSGAGSGTHFTLIISTLQPEDSATYYCQQSYSTPWTFGQGTKVEIK

SEQ ID NO: 21 - DNA, 385 bp, homo sapiens
gatgtgcagttggtggagtctgggggaggcgtggtccagccgggggggtccctgaaactcgcctgtgtagtctctggattcaggtttagtgactactggatgagttgggtccgccaggccccagggaaggggctggaatgggtggccaacataaaacaagatggaagtgggaagtactatgtggactccgtgaagggccgattcaccgtctccagagacaacgccaagaactcactgtatctacacatgaccagcctgggagccgaggacacggccgtatacttctgcgcgagagcagcccccaccggctcctacactaatatcctagtcgacaacgtccacttcgactactggggccagggaatcctggtcgccgtctcctcag

SEQ ID NO: 22 - DNA, 322 bp, homo sapiens
ggcatccagctgacccagtctccaggctccctgtctgcatctgtaggagacagtgtcaccatcacttgccggccaaatcagaacatcgccacctatataaattggtatcagcagacaccagggaaagcccctaagctcctgatctatgccgcatccattttgcagagtggggtcccatcaaggttcagtggcgctggatctgggacacatttcactctcatcatcagtaccctacaacctgaggattctgcaacttactactgccaacagagttacagtaccccgtggacattcggccaagggaccaaagtggaaatcaaac

SEQ ID NO: 23 - protein, 113 aa, homo sapiens
AVQLVQSGAEVKKPGTTVKISCKVSGYTFIQEYIHWVQQAPGKGLVWMGLGDPENNETLYSEDFQGRVTMTADTSSDTAYLELRSLTFADTAVYFCTSRKSWWGQGTLVTVAS

SEQ ID NO: 24 - protein, 111 aa, homo sapiens
ELVLTQSPGTLSLSPGESATLSCRASQSLSSDSVSWFQQKPGQAPRLVIHGTSKRATGIPDRFSGGGSGTDFTLTIARLEPEDFAVYYCQRSGYGMSVTWTFGQGTTVEIK

SEQ ID NO: 25 - DNA, 340 bp, homo sapiens
gcggtccagttggtacaatctggggctgaggtgaagaagcctgggaccaccgtcaaaatctcctgcaaagtttctggatacaccttcattcaagaatacatacactgggtgcaacaggcccctggaaaagggcttgtgtggatgggacttggtgaccctgaaaataatgagactctatattcagaggatttccaaggcagagtcaccatgaccgcggacacatcctcagacacagcctatctggaactgcgcagcctgacatttgcagacacggccgtctatttctgtacatcacgaaagtcctggtggggccagggaaccctggtcaccgtcgcctcag

SEQ ID NO: 26 - DNA, 334 bp, homo sapiens
gaacttgtgttgacgcagtctccaggcaccctgtctttgtctccaggggaaagcgccaccctctcctgtagggccagtcagagtcttagcagcgactctgtatcttggttccagcagaaacctggccaggctcccaggctcgtcatccatggtacatcaaagagggccactggcatcccagacaggttcagtggcggtgggtctgggacagacttcactctcaccatcgccagactggagcctgaggattttgcagtctattattgtcagcggtctgggtatggtatgtcagtcacgtggacgttcggccaagggaccacggtggagatcaaac

SEQ ID NO: 27 - DNA, 334 bp, homo sapiens
gaacttgtgttgacgcagtctccaggcaccctgtctttgtctccaggggaaagcgccaccctctcctgtagggccagtcagagtcttagcagcgactctgtatcttggttccagcagaaacctggccaggctcccaggctcgtcatccatggtacatcaaagagggccactggcatcccagacaggttcagtggcggtgggtctgggacagacttcactctcaccatcgccagactggagcctgaggattttgcagtctattattgtcagcggtctgggtatggtatgtcagtcacgtggacgtttggccaagggaccacggtggagatcaaac

SEQ ID NO: 28 - protein, 119 aa, homo sapiens
EVQLVESGGGLIQPGGSLRLSCAASGFALRSYDMHWVRQTIDKRLEWVSAVGPSGDTYYADSVKGRFAVSRENAKNSLSLQMNSLTAGDTAIYYCVRSDRGVAGLFDSWGQGILVTVSS

SEQ ID NO: 29 - protein, 106 aa, homo sapiens
DIQMTQSPSSLSASVGDRITITCRASQAFSNYVAWYQQRPGKVPKLLISAASALHAGVPSRFSGSGSGTHFTLTISSLQPEDVATYYCQNYNSAPLTFGGGTKVEI

SEQ ID NO: 30 - DNA, 357 bp, homo sapiens
gaagtgcagctggtggagtctggaggaggtctgattcagcccgggggttccctgcgtctgagttgtgccgcatctggatttgctctgcgaagctacgacatgcactgggtgagacagactatcgataagcgcctggagtgggtgtctgctgtcggccccagtggagacacctactatgcagattcagtgaaggggaggttcgcagtctcccgggaaaacgccaaaaattccctgagcctgcagatgaactctctgaccgccggcgacacagctatctactattgcgtcaggagcgatagaggggtcgcaggactgtttgattcatggggtcagggtattctggtcaccgtgtcttca

SEQ ID NO: 31 - DNA, 318 bp, homo sapiens
gatattcagatgactcagagcccttcctcactgtccgcatccgtgggagaccgtattactattacttgtagagcttctcaggctttttctaactacgtggcttggtatcagcagaggcccggcaaggtccctaaactgctgatctccgccgcttctgcactgcatgctggagtgccaagccggttctctggaagtggatcagggactcacttcaccctgacaatttccagcctgcagcccgaggatgtcgcaacctactattgccagaactacaacagtgctcccctgacattcggtggtggaacaaaggtcgagatc

SEQ ID NO: 32 - protein, 8 aa, homo sapiens
GFALRMYD

SEQ ID NO: 33 - protein, 7 aa, homo sapiens
VGPSGDT

SEQ ID NO: 34 - protein, 13 aa, homo sapiens
VRSDRGVAGLFDS

SEQ ID NO: 35 - protein, 6 aa, homo sapiens
QAFDNY

SEQ ID NO: 36 - protein, 3 aa, homo sapiens
AAS

SEQ ID NO: 37 - protein, 9 aa, homo sapiens
QNYNSAPLT

SEQ ID NO: 38 - protein, 8 aa, homo sapiens
GFALRSYD

SEQ ID NO: 39 - protein, 6 aa, homo sapiens
QAFSNY

SEQ ID NO: 40 - protein, 8 aa, homo sapiens
GGSLSSFY

SEQ ID NO: 41 - protein, 7 aa, homo sapiens
IYYSGSP

SEQ ID NO: 42 - protein, 19 aa, homo sapiens
VRASRSYYWGSYRPTAFDS

SEQ ID NO: 43 - protein, 6 aa, homo sapiens
NLGDKY

SEQ ID NO: 44 - protein, 3 aa, homo sapiens
QDN

SEQ ID NO: 45 - protein, 8 aa, homo sapiens
QTWDSTVV

SEQ ID NO: 46 - protein, 8 aa, homo sapiens
GFRFSDYW

SEQ ID NO: 47 - protein, 8 aa, homo sapiens
IKQDGSGK

SEQ ID NO: 48 - protein, 21 aa, homo sapiens
ARAAPTGSYTNILVDNVHFDY

SEQ ID NO: 49 - protein, 6 aa, homo sapiens
QNIATY

SEQ ID NO: 50 - protein, 9 aa, homo sapiens
QQSYSTPWT

SEQ ID NO: 51 - protein, 8 aa, homo sapiens
GGTLSNYA

SEQ ID NO: 52 - protein, 8 aa, homo sapiens
TIPTLGMS

SEQ ID NO: 53 - protein, 16 aa, homo sapiens
ATMGSADTSFYFYMDV

SEQ ID NO: 54 - protein, 7 aa, homo sapiens
QSVSSSY

SEQ ID NO: 55 - protein, 3 aa, homo sapiens
GTS

SEQ ID NO: 56 - protein, 9 aa, homo sapiens
QQYAYSPFT

SEQ ID NO: 57 - protein, 8 aa, homo sapiens
GYTFIQEY

SEQ ID NO: 58 - protein, 8 aa, homo sapiens
GDPENNET

SEQ ID NO: 59 - protein, 6 aa, homo sapiens
TSRKSW

SEQ ID NO: 60 - protein, 7 aa, homo sapiens
QSLSSDS

SEQ ID NO: 61 - protein, 12 aa, homo sapiens
QRSGYGMSVTWT

SEQ ID NO: 62 - protein, 108 aa, homo sapiens
EIVLTQSPGTLSLSPGERATLSCRASQSVSSSYLAWYQQKPGQAPRLLIYGTSSRATGIPDRFSGSASGTDFTLTISRLEPEDFAVYYCQQYAYSPFTFGPGTTVDIK

SEQ ID NO: 63 - DNA, 23 bp, Artificial sequence
  DNA primer
ttttcaatcctcaaccgtaaggc

SEQ ID NO: 64 - DNA, 20 bp, Artificial sequence
  DNA primer
cagtccggtcccagaatgtg

SEQ ID NO: 65 - DNA, 21 bp, Artificial sequence
  DNA primer
catgtgccgccccatcgctgc

SEQ ID NO: 66 - protein, 58 aa, Artificial sequence
  Modified Ebola virus GP
MKQIEDKIEEILSKIYHIENEIARIKKLIGEVASSSIEGRGSHHHHHHSAWSHPQFEK